European Patent Application EP 4 681 725 A1, published January 21, 2026. Title: 心肥大の治療薬及び検査方法. Applicant: 学校法人東海大学. The sequence listing filed with the application follows.

SEQUENCE LISTING (45 sequences)

SEQ ID NO: 1 - protein, 202 aa, Homo sapiens
MLVAGFLLALPPSWAAGAPRAGRRPARPRGCADRPEELLEQLYGRLAAGVLSAFHHTLQLGPREQARNASCPAGGRPADRRFRPPTNLRSVSPWAYRISYDPARYPRYLPEAYCLCRGCLTGLFGEEDVRFRSAPVYMPTVVLRRTPACAGGRSVYTEAYVTIPVGCTCVPEPEKDADSINSSIDKQGAKLLLGPNDAPAGP

SEQ ID NO: 2 - protein, 202 aa, Pongo abelii
MLVAGFLLALPPGGAAGAPRAGRRPARPRGCADRPEELLEQLYGRLAAGVLSAFHHTLQLGPREQARNASCPAGGRPADRRFRPPTNLRSVSPWAYRISYDPARYPRYLPEAYCLCRGCLTGLFGEEDVRFRSAPVYMPTVVLRRTPACAGGRSVYTEAYVTIPVGCTCVPEPEKDADSINSSIDKQGAKLLLGPNHAPAGP

SEQ ID NO: 3 - protein, 192 aa, Bos taurus
VWALVAGVLLALSPGRAGGAPKAGRRPARARGCADRPEELLEQLYGRLAAGVLGAFHHTLQLGPREQARNASCPAGGRPADRRFRPPTNLRSVSPWAYRISYDPGRFPRYLPEAYCLCRGCLTGPRGEEDVRLRSAPVLVPAVVLRRTPGCAGGRAVYVEEYVTVPVGCTCVPGPDKDADAANSSLDKSARP

SEQ ID NO: 4 - protein, 193 aa, Capra hircus
MVWALVAGVLLALSPGRAGGAPKAGRRPARARGCADRPEELLEQLYGRLAAGVLGAFHHTLQLGPREQARNASCPAGGRPADRRFRPPTNLRSVSPWAYRISYDPGRFPRYLPEAYCLCRGCLTGPRGEEDVRLRSAPVLVPAVVLRRTPGCAGGRAVYVEEYVTVPVGCTCVPGPDKDADAVNSSLDKSARP

SEQ ID NO: 5 - protein, 202 aa, Felis catus
MLAVGVLLALAPGRAAGALRASRRPARPRGCAERPEELLEQLYGRLAAGVLGAFHHTLQLGPREQARNASCPAGGRPGDRRFRPPTNLRSVSPWAYRISYDPARYPKYLPEAYCLCRGCLTGLFGEEDLRFRSAPVYMPTVILRRTSACAGGRWVYTEEYVTVPVGCTCVPEQEKEADAVNSSMDKQGARLLLGPGDKPGRP

SEQ ID NO: 6 - protein, 205 aa, Rattus norvegicus
MLGTLVWMPSSAPVALAPGRAAGAARKGXAARPRDCADRPRSSLEQLYGGWPAGLPAPSHQHLQLGPREQARNATLPGRGRSXDRRFRPRHHLRSRCPPLGPYRISYDPARFPRYLPEAYCLCRGCLTGLYGEEDFRFRSAPVFSPAVVLRRTAACAGGRSVYAEHYITIPVGCTCVPEPDKSADSANSSMDKMLLGVADRPAGR

SEQ ID NO: 7 - protein, 205 aa, Mus musculus
MLGTLVWMLAVGFLLALAPGRAAGALRTGRRPARPRDCADRPEELLEQLYGRLAAGVLSAFHHTLQLGPREQARNASCPAGGRAADRRFRPPTNLRSVSPWAYRISYDPARFPRYLPEAYCLCRGCLTGLYGEEDFRFRSTPVFSPAVVLRRTAACAGGRSVYAEHYITIPVGCTCVPEPDKSADSANSSMDKLLLGPADRPAGR

SEQ ID NO: 8 - protein, 216 aa, Xenopus laevis
MKSNSKVWILKAALMLLFGILIASCDGSKPVKRPPPKPRNCADRPEEHLELVYGRLAAGMLSAYHHTLQLQPLDKENISCPAGTQGGGAVDGKQRLPVNIHSISPWAYRISYNPTRYPKYIPEAYCLCKGCLTGPLGEENFHFRSLPVYMPTVILRRTSTCAGGRYVYEEEYITIPVGCTCVPEQEKGAESESVNSSLEKEKFKLPLNKSEKPLVN

SEQ ID NO: 9 - protein, 212 aa, Danio rerio
MRAPVVSTLVLVWLWCCGSAPGERGQKVSRRAPRTRSCLDLPEEILEQMFGRLSVGVLSAFHHTLQLATPERQNLSCGSASRLARDRPRTPVNLLSLSPWAYRISHDPARYPRYLPEAYCLCKGCLSGLNGEESDRFRSTPVYMPTVILRRTVGPCVGGRHSYTESYVSIAVGCTCVPLLEKDSKIQKSKPSVRRVASKNTVSSTFRKNELN

SEQ ID NO: 10 - protein, 253 aa, Homo sapiens
MLVAGFLLALPPSWAAGAPRAGRRPARPRGCADRPEELLEQLYGRLAAGVLSAFHHTLQLGPREQARNASCPAGGRPADRRFRPPTNLRSVSPWAYRISYDPARYPRYLPEAYCLCRGCLTGLFGEEDVRFRSAPVYMPTVVLRRTPACAGGRSVYTEAYVTIPVGCTCVPEPEKDADSINSSIDKQGAKLLLGPNDAPAGPCGRSCPGRSPRPASRGAQAGAAWRARSATSEESAPSKPSAGAPAPPFHGDS

SEQ ID NO: 11 - DNA, 57 bp, Mus musculus
  source 1..57: mol_type = genomic DNA
ctgctggggcccgccgacaggcctgcggggcgctgatgccggggactgcccgccatg

SEQ ID NO: 12 - DNA, 19 bp, synthetic construct
  source 1..19: mol_type = other DNA
ctgctgggggcccgccatg

SEQ ID NO: 13 - protein, 212 aa, synthetic construct
MLGTLVWMLAVGFLLALAPGRAAGALRTGRRPARPRDCADRPEELLEQLYGRLAAGVLSAFHHTLQLGPREQARNASCPAGGRAADRRFRPPTNLRSVSPWAYRISYDPARFPRYLPEAYCLCRGCLTGLYGEEDFRFRSTPVFSPAVVLRRTAACAGGRSVYAEHYITIPVGCTCVPEPDKSADSANSSMDKLLLGARHGPASCMHQVPWP

SEQ ID NO: 14 - DNA, 24 bp, Rattus norvegicus
  source 1..24: mol_type = genomic DNA
aggccggcggggcgctgatgagac

SEQ ID NO: 15 - DNA, 22 bp, synthetic construct
  source 1..22: mol_type = other DNA
aggccggcggcgctgatgagac

SEQ ID NO: 16 - DNA, 19 bp, synthetic construct
  source 1..19: mol_type = other DNA
tcccatcctccggccgcct

SEQ ID NO: 17 - DNA, 20 bp, synthetic construct
  source 1..20: mol_type = other DNA
gccaaccacctccttccccg

SEQ ID NO: 18 - DNA, 19 bp, synthetic construct
  source 1..19: mol_type = other DNA
tccccgtgactctaaccag

SEQ ID NO: 19 - DNA, 18 bp, synthetic construct
  source 1..18: mol_type = other DNA
cactcttcaggagtcgcc

SEQ ID NO: 20 - DNA, 23 bp, synthetic construct
  source 1..23: mol_type = other DNA
gctgtgttcccatccatcatcgt

SEQ ID NO: 21 - DNA, 20 bp, synthetic construct
  source 1..20: mol_type = other DNA
gtcaggatacctcgcttgct

SEQ ID NO: 22 - DNA, 18 bp, synthetic construct
  source 1..18: mol_type = other DNA
atcgctgcgctcgtcgtc

SEQ ID NO: 23 - DNA, 20 bp, synthetic construct
  source 1..20: mol_type = other DNA
cttctgacccatacccacca

SEQ ID NO: 24 - DNA, 17 bp, synthetic construct
  source 1..17: mol_type = other DNA
gctgagacagaatgcaa

SEQ ID NO: 25 - DNA, 19 bp, synthetic construct
  source 1..19: mol_type = other DNA
cctgatcttgtcgaacttg

SEQ ID NO: 26 - DNA, 26 bp, synthetic construct
  source 1..26: mol_type = other DNA
atgttgggactggtctggatgcctcg

SEQ ID NO: 27 - DNA, 22 bp, synthetic construct
  source 1..22: mol_type = other DNA
tcagcgccgccgccgcctgtca

SEQ ID NO: 28 - DNA, 22 bp, synthetic construct
  source 1..22: mol_type = other DNA
ccggcagtctcatcagcgccgc

SEQ ID NO: 29 - DNA, 22 bp, synthetic construct
  source 1..22: mol_type = other DNA
aaacgcggcgctgatgagactg

SEQ ID NO: 30 - DNA, 18 bp, synthetic construct
  source 1..18: mol_type = other DNA
aagcctactgcctgccga

SEQ ID NO: 31 - DNA, 20 bp, synthetic construct
  source 1..20: mol_type = other DNA
tggatggatctggtgtgctt

SEQ ID NO: 32 - DNA, 23 bp, synthetic construct
  source 1..23: mol_type = other DNA
ccggggagcagctgtacggcgcc

SEQ ID NO: 33 - DNA, 23 bp, synthetic construct
  source 1..23: mol_type = other DNA
aaacggccccgtacagctgctcc

SEQ ID NO: 34 - DNA, 23 bp, synthetic construct
  source 1..23: mol_type = other DNA
ccggcctgcgagcgtgtcgccct

SEQ ID NO: 35 - DNA, 23 bp, synthetic construct
  source 1..23: mol_type = other DNA
aaacaggcgacacgctgcgcagg

SEQ ID NO: 36 - DNA, 24 bp, synthetic construct
  source 1..24: mol_type = other DNA
ccggcaactccagcatcgacaaac

SEQ ID NO: 37 - DNA, 24 bp, synthetic construct
  source 1..24: mol_type = other DNA
aaacgtttgtcgatgctggagttg

SEQ ID NO: 38 - DNA, 36 bp, synthetic construct
  source 1..36: mol_type = other DNA
ccggcatcagcgccgcgtttagagctatgctgtttg

SEQ ID NO: 39 - DNA, 61 bp, synthetic construct
  source 1..61: mol_type = other DNA
aaacagcatagcaagttaaaaaggctagtccgttacaactgaaaaggcaccgagtcgtgct

SEQ ID NO: 40 - DNA, 20 bp, synthetic construct
  source 1..20: mol_type = other DNA
aggaggacttccgctttcgc

SEQ ID NO: 41 - DNA, 20 bp, synthetic construct
  source 1..20: mol_type = other DNA
aggaggacttccgctttcgc

SEQ ID NO: 42 - DNA, 24 bp, synthetic construct
  source 1..24: mol_type = other DNA
ccggcaatgactgcgtaagatccc

SEQ ID NO: 43 - DNA, 24 bp, synthetic construct
  source 1..24: mol_type = other DNA
aaacgggatcttacgcagtcattg

SEQ ID NO: 44 - DNA, 24 bp, synthetic construct
  source 1..24: mol_type = other DNA
ccggtgcacactcaccgcccgatg

SEQ ID NO: 45 - DNA, 24 bp, synthetic construct
  source 1..24: mol_type = other DNA
aaaccatcgggcggtgagtgtgca